European Patent Specification EP 2 956 174 B1, published October 15, 2025. Title: METHODS AND COMPOSITIONS FOR TREATING GENETICALLY LINKED DISEASES OF THE EYE. Applicant: The United States of America, as represented by the Secretary, Department of Health and Human Services Colosi, Peter Sieving, Paul Albert Zeng, Yong Bush, Ronald Avery. Application not yet assigned. The sequence listing filed with the application follows.

SEQUENCE LISTING (16 sequences)

SEQ ID NO: 1 - DNA, 675 bp, Homo sapien
atgtcacgcaagatagaaggctttttgttattacttctctttggctatgaagccacattgggattatcgtctaccgaggatgaaggcgaggacccctggtaccaaaaagcatgcaagtgcgattgccaaggaggacccaatgctctgtggtctgcaggtgccacctccttggactgtataccagaatgcccatatcacaagcctctgggtttcgagtcaggggaggtcacaccggaccagatcacctgctctaacccggagcagtatgtgggctggtattcttcgtggactgcaaacaaggcccggctcaacagtcaaggctttgggtgtgcctggctctccaagttccaggacagtagccagtggttacagatagatctgaaggagatcaaagtgatttcagggatcctcacccaggggcgctgtgacatcgatgagtggatgaccaagtacagcgtgcagtacaggaccgatgagcgcctgaactggatttactacaaggaccagactggaaacaaccgggtcttctatggcaactcggaccgcacctccacggttcagaacctgctgcggccccccatcatctcccgcttcatccgcctcatcccgctgggctggcacgtccgcattgccatccggatggagctgctggagtgcgtcagcaagtgtgcctga

SEQ ID NO: 2 - protein, 224 aa, Homo sapien
MSRKIEGFLLLLLFGYEATLGLSSTEDEGEDPWYQKACKCDCQGGPNALWSAGATSLDCIPECPYHKPLGFESGEVTPDQITCSNPEQYVGWYSSWTANKARLNSQGFGCAWLSKFQDSSQWLQIDLKEIKVISGILTQGRCDIDEWMTKYSVQYRTDERLNWIYYKDQTGNNRVFYGNSDRTSTVQNLLRPPIISRFIRLIPLGWHVRIAIRMELLECVSKCA

SEQ ID NO: 3 - DNA, 675 bp, Homo sapien
tcaggcacacttgctgacgcactccagcagctccatccggatggcaatgcggacgtgccagcccagcgggatgaggcggatgaagcgggagatgatggggggccgcagcaggttctgaaccgtggaggtgcggtccgagttgccatagaagacccggttgtttccagtctggtccttgtagtaaatccagttcaggcgctcatcggtcctgtactgcacgctgtacttggtcatccactcatcgatgtcacagcgcccctgggtgaggatccctgaaatcactttgatctccttcagatctatctgtaaccactggctactgtcctggaacttggagagccaggcacacccaaagccttgactgttgagccgggccttgtttgcagtccacgaagaataccagcccacatactgctccgggttagagcaggtgatctggtccggtgtgacctcccctgactcgaaacccagaggcttgtgatatgggcattctggtatacagtccaaggaggtggcacctgcagaccacagagcattgggtcctccttggcaatcgcacttgcatgctttttggtaccaggggtcctcgccttcatcctcggtagacgataatcccaatgtggcttcatagccaaagagaagtaataacaaaaagccttctatcttgcgtgacat

SEQ ID NO: 4 - DNA, 606 bp, Homo sapien
tctaccgaggatgaaggcgaggacccctggtaccaaaaagcatgcaagtgcgattgccaaggaggacccaatgctctgtggtctgcaggtgccacctccttggactgtataccagaatgcccatatcacaagcctctgggtttcgagtcaggggaggtcacaccggaccagatcacctgctctaacccggagcagtatgtgggctggtattcttcgtggactgcaaacaaggcccggctcaacagtcaaggctttgggtgtgcctggctctccaagttccaggacagtagccagtggttacagatagatctgaaggagatcaaagtgatttcagggatcctcacccaggggcgctgtgacatcgatgagtggatgaccaagtacagcgtgcagtacaggaccgatgagcgcctgaactggatttactacaaggaccagactggaaacaaccgggtcttctatggcaactcggaccgcacctccacggttcagaacctgctgcggccccccatcatctcccgcttcatccgcctcatcccgctgggctggcacgtccgcattgccatccggatggagctgctggagtgcgtcagcaagtgtgcctga

SEQ ID NO: 5 - protein, 201 aa, Homo sapien
STEDEGEDPWYQKACKCDCQGGPNALWSAGATSLDCIPECPYHKPLGFESGEVTPDQITCSNPEQYVGWYSSWTANKARLNSQGFGCAWLSKFQDSSQWLQIDLKEIKVISGILTQGRCDIDEWMTKYSVQYRTDERLNWIYYKDQTGNNRVFYGNSDRTSTVQNLLRPPIISRFIRLIPLGWHVRIAIRMELLECVSKCA

SEQ ID NO: 6 - DNA, 606 bp, Homo sapien
tcaggcacacttgctgacgcactccagcagctccatccggatggcaatgcggacgtgccagcccagcgggatgaggcggatgaagcgggagatgatggggggccgcagcaggttctgaaccgtggaggtgcggtccgagttgccatagaagacccggttgtttccagtctggtccttgtagtaaatccagttcaggcgctcatcggtcctgtactgcacgctgtacttggtcatccactcatcgatgtcacagcgcccctgggtgaggatccctgaaatcactttgatctccttcagatctatctgtaaccactggctactgtcctggaacttggagagccaggcacacccaaagccttgactgttgagccgggccttgtttgcagtccacgaagaataccagcccacatactgctccgggttagagcaggtgatctggtccggtgtgacctcccctgactcgaaacccagaggcttgtgatatgggcattctggtatacagtccaaggaggtggcacctgcagaccacagagcattgggtcctccttggcaatcgcacttgcatgctttttggtaccaggggtcctcgccttcatcctcggtaga

SEQ ID NO: 7 - DNA, 489 bp, Homo sapien
tgcccatatcacaagcctctgggtttcgagtcaggggaggtcacaccggaccagatcacctgctctaacccggagcagtatgtgggctggtattcttcgtggactgcaaacaaggcccggctcaacagtcaaggctttgggtgtgcctggctctccaagttccaggacagtagccagtggttacagatagatctgaaggagatcaaagtgatttcagggatcctcacccaggggcgctgtgacatcgatgagtggatgaccaagtacagcgtgcagtacaggaccgatgagcgcctgaactggatttactacaaggaccagactggaaacaaccgggtcttctatggcaactcggaccgcacctccacggttcagaacctgctgcggccccccatcatctcccgcttcatccgcctcatcccgctgggctggcacgtccgcattgccatccggatggagctgctggagtgcgtcagcaagtgtgcctga

SEQ ID NO: 8 - protein, 162 aa, Homo sapien
CPYHKPLGFESGEVTPDQITCSNPEQYVGWYSSWTANKARLNSQGFGCAWLSKFQDSSQWLQIDLKEIKVISGILTQGRCDIDEWMTKYSVQYRTDERLNWIYYKDQTGNNRVFYGNSDRTSTVQNLLRPPIISRFIRLIPLGWHVRIAIRMELLECVSKCA

SEQ ID NO: 9 - DNA, 1071 bp, Artificial Sequence
  Human retinoschisin promoter construct
gcggccgcaccaccaaatttagcattttcctgagtgaataggtgtgcacatgatgcctagttgctttcaaagaggggaatccatgacattttcatacaattcgagaatgttagtgcttatgtggcaggaaattgttcaaggtcaccccctaaaaaatgatggcgaagaaaggacgaaaacctgagacttctggttgtagttctctccctccattgcttcccttacattaagatagaatgaacagtatggtcgacggcccaggcttcccagcagggctaaggatatgcaaggagtgcattcatccggaggtgttggcagcatcccagccccaccccattctcatcgtaaatcaggctcacttccattggctgcatacggtggagtgatgtgaccatatgtcacttgagcattacacaaatcctaatgagctaaaaatatgtttgttttagctaattgacctctttggccttcataaagcagttggtaaacatcctcagataatgatttccaaagaggtcgaccgaaaagtatcttcctcgcgaactgaatctcagttgatgctagtatcttccatgagacttccttgttgaggcaggtaactctgtgggttaacttgatggggctcagccaaagacctaagaactaaatggattaagatgcttaatgaggccagggctcaacttaatcccctgctcctgggccagctctccagttcagtaaggtagagctttggccgaggacgaggggaagatgtcacgcaagatagaaggctttttgttattacttctctttggctatgaaggtatgtgctattcaaccattgacattcattgcatacttaatacataatttaattaatatcgttgataaataggaatatagcctgaataatataaatattattaattagcaacacgttaattaactaacatgtgttattaatgaacaacagttgtctttgtgtggatggctttccagttctgtgaggagccttctaaagttcaaaggatgcttaaaatccaacagaaaacaggatgggtctcagaaatctataaaatagccagcgatcgc

SEQ ID NO: 10 - DNA, 245 bp, Homo sapien
aagatagaaggctttttgttattacttctctttggctatgaagccacattgggattatcgtctaccgaggatgaaggcgaggacccctggtaccaaaaagcatgcaagtgcgattgccaaggaggacccaatgctctgtggtctgcaggtgccacctccttggactgtataccagaatgcccatatcacaagcctctgggtttcgagtcaggggaggtcacaccggaccagatcacctgctctaa

SEQ ID NO: 11 - DNA, 229 bp, Artificial Sequence
  Human retinoschisin promoter sequence (nucleotides 522-750 of SEQ ID NO:9)
cgaaaagtatcttcctcgcgaactgaatctcagttgatgctagtatcttccatgagacttccttgttgaggcaggtaactctgtgggttaacttgatggggctcagccaaagacctaagaactaaatggattaagatgcttaatgaggccagggctcaacttaatcccctgctcctgggccagctctccagttcagtaaggtagagctttggccgaggacgaggggaag

SEQ ID NO: 12 - DNA, 261 bp, Homo sapien
ggcccaggcttcccagcagggctaaggatatgcaaggagtgcattcatccggaggtgttggcagcatcccagccccaccccattctcatcgtaaatcaggctcacttccattggctgcatacggtggagtgatgtgaccatatgtcacttgagcattacacaaatcctaatgagctaaaaatatgtttgttttagctaattgacctctttggccttcataaagcagttggtaaacatcctcagataatgatttccaaagag

SEQ ID NO: 13 - DNA, 2217 bp, Adeno-associated virus
atggctgccgatggttatcttccagattggctcgaggacaacctctctgagggcattcgcgagtggtgggcgctgaaacctggagccccgaagcccaaagccaaccagcaaaagcaggacgacggccggggtctggtgcttcctggctacaagtacctcggacccttcaacggactcgacaagggggagcccgtcaacgcggcggacgcagcggccctcgagcacgacaaggcctacgaccagcagctgcaggcgggtgacaatccgtacctgcggtataaccacgccgacgccgagtttcaggagcgtctgcaagaagatacgtcttttgggggcaacctcgggcgagcagtcttccaggccaagaagcgggttctcgaacctctcggtctggttgaggaaggcgctaagacggctcctggaaagaagagaccggtagagccatcaccccagcgttctccagactcctctacgggcatcggcaagaaaggccaacagcccgccagaaaaagactcaattttggtcagactggcgactcagagtcagttccagaccctcaacctctcggagaacctccagcagcgccctctggtgtgggacctaatacaatggctgcaggcggtggcgcaccaatggcagacaataacgaaggcgccgacggagtgggtagttcctcgggaaattggcattgcgattccacatggctgggcgacagagtcatcaccaccagcacccgaacctgggccctgcccacctacaacaaccacctctacaagcaaatctccaacgggacatcgggaggagccaccaacgacaacacctacttcggctacagcaccccctgggggtattttgactttaacagattccactgccacttttcaccacgtgactggcagcgactcatcaacaacaactggggattccggcccaagagactcagcttcaagctcttcaacatccaggtcaaggaggtcacgcagaatgaaggcaccaagaccatcgccaataacctcaccagcaccatccaggtgtttacggactcggagtaccagctgccgtacgttctcggctctgcccaccagggctgcctgcctccgttcccggcggacgtgttcatgattccccagtacggctacctaacactcaacaacggtagtcaggccgtgggacgctcctccttctactgcctggaatactttccttcgcagatgctgagaaccggcaacaacttccagtttacttacaccttcgaggacgtgcctttccacagcagctacgcccacagccagagcttggaccggctgatgaatcctctgattgaccagtacctgtactacttgtctcggactcaaacaacaggaggcacggcaaatacgcagactctgggcttcagccaaggtgggcctaatacaatggccaatcaggcaaagaactggctgccaggaccctgttaccgccaacaacgcgtctcaacgacaaccgggcaaaacaacaatagcaactttgcctggactgctgggaccaaataccatctgaatggaagaaattcattggctaatcctggcatcgctatggcaacacacaaagacgacgaggagcgtttttttcccagtaacgggatcctgatttttggcaaacaaaatgctgccagagacaatgcggattacagcgatgtcatgctcaccagcgaggaagaaatcaaaaccactaaccctgtggctacagaggaatacggtatcgtggcagataacttgcagcagcaaaacacggctcctcaaattggaactgtcaacagccagggggccttacccggtatggtctggcagaaccgggacgtgtacctgcagggtcccatctgggccaagattcctcacacggacggcaacttccacccgtctccgctgatgggcggctttggcctgaaacatcctccgcctcagatcctgatcaagaacacgcctgtacctgcggatcctccgaccaccttcaaccagtcaaagctgaactctttcatcacgcaatacagcaccggacaggtcagcgtggaaattgaatgggagctgcagaaggaaaacagcaagcgctggaaccccgagatccagtacacctccaactactacaaatctacaagtgtggactttgctgttaatacagaaggcgtgtactctgaaccccgccccattggcacccgttacctcacccgtaatctgtaa

SEQ ID NO: 14 - protein, 738 aa, Adeno-associated virus
MAADGYLPDWLEDNLSEGIREWWALKPGAPKPKANQQKQDDGRGLVLPGYKYLGPFNGLDKGEPVNAADAAALEHDKAYDQQLQAGDNPYLRYNHADAEFQERLQEDTSFGGNLGRAVFQAKKRVLEPLGLVEEGAKTAPGKKRPVEPSPQRSPDSSTGIGKKGQQPARKRLNFGQTGDSESVPDPQPLGEPPAAPSGVGPNTMAAGGGAPMADNNEGADGVGSSSGNWHCDSTWLGDRVITTSTRTWALPTYNNHLYKQISNGTSGGATNDNTYFGYSTPWGYFDFNRFHCHFSPRDWQRLINNNWGFRPKRLSFKLFNIQVKEVTQNEGTKTIANNLTSTIQVFTDSEYQLPYVLGSAHQGCLPPFPADVFMIPQYGYLTLNNGSQAVGRSSFYCLEYFPSQMLRTGNNFQFTYTFEDVPFHSSYAHSQSLDRLMNPLIDQYLYYLSRTQTTGGTANTQTLGFSQGGPNTMANQAKNWLPGPCYRQQRVSTTTGQNNNSNFAWTAGTKYHLNGRNSLANPGIAMATHKDDEERFFPSNGILIFGKQNAARDNADYSDVMLTSEEEIKTTNPVATEEYGIVADNLQQQNTAPQIGTVNSQGALPGMVWQNRDVYLQGPIWAKIPHTDGNFHPSPLMGGFGLKHPPPQILIKNTPVPADPPTTFNQSKLNSFITQYSTGQVSVEIEWELQKENSKRWNPEIQYTSNYYKSTSVDFAVNTEGVYSEPRPIGTRYLTRNL

SEQ ID NO: 15 - DNA, 2217 bp, Homo sapien
ttacagattacgggtgaggtaacgggtgccaatggggcggggttcagagtacacgccttctgtattaacagcaaagtccacacttgtagatttgtagtagttggaggtgtactggatctcggggttccagcgcttgctgttttccttctgcagctcccattcaatttccacgctgacctgtccggtgctgtattgcgtgatgaaagagttcagctttgactggttgaaggtggtcggaggatccgcaggtacaggcgtgttcttgatcaggatctgaggcggaggatgtttcaggccaaagccgcccatcagcggagacgggtggaagttgccgtccgtgtgaggaatcttggcccagatgggaccctgcaggtacacgtcccggttctgccagaccataccgggtaaggccccctggctgttgacagttccaatttgaggagccgtgttttgctgctgcaagttatctgccacgataccgtattcctctgtagccacagggttagtggttttgatttcttcctcgctggtgagcatgacatcgctgtaatccgcattgtctctggcagcattttgtttgccaaaaatcaggatcccgttactgggaaaaaaacgctcctcgtcgtctttgtgtgttgccatagcgatgccaggattagccaatgaatttcttccattcagatggtatttggtcccagcagtccaggcaaagttgctattgttgttttgcccggttgtcgttgagacgcgttgttggcggtaacagggtcctggcagccagttctttgcctgattggccattgtattaggcccaccttggctgaagcccagagtctgcgtatttgccgtgcctcctgttgtttgagtccgagacaagtagtacaggtactggtcaatcagaggattcatcagccggtccaagctctggctgtgggcgtagctgctgtggaaaggcacgtcctcgaaggtgtaagtaaactggaagttgttgccggttctcagcatctgcgaaggaaagtattccaggcagtagaaggaggagcgtcccacggcctgactaccgttgttgagtgttaggtagccgtactggggaatcatgaacacgtccgccgggaacggaggcaggcagccctggtgggcagagccgagaacgtacggcagctggtactccgagtccgtaaacacctggatggtgctggtgaggttattggcgatggtcttggtgccttcattctgcgtgacctccttgacctggatgttgaagagcttgaagctgagtctcttgggccggaatccccagttgttgttgatgagtcgctgccagtcacgtggtgaaaagtggcagtggaatctgttaaagtcaaaatacccccagggggtgctgtagccgaagtaggtgttgtcgttggtggctcctcccgatgtcccgttggagatttgcttgtagaggtggttgttgtaggtgggcagggcccaggttcgggtgctggtggtgatgactctgtcgcccagccatgtggaatcgcaatgccaatttcccgaggaactacccactccgtcggcgccttcgttattgtctgccattggtgcgccaccgcctgcagccattgtattaggtcccacaccagagggcgctgctggaggttctccgagaggttgagggtctggaactgactctgagtcgccagtctgaccaaaattgagtctttttctggcgggctgttggcctttcttgccgatgcccgtagaggagtctggagaacgctggggtgatggctctaccggtctcttctttccaggagccgtcttagcgccttcctcaaccagaccgagaggttcgagaacccgcttcttggcctggaagactgctcgcccgaggttgcccccaaaagacgtatcttcttgcagacgctcctgaaactcggcgtcggcgtggttataccgcaggtacggattgtcacccgcctgcagctgctggtcgtaggccttgtcgtgctcgagggccgctgcgtccgccgcgttgacgggctcccccttgtcgagtccgttgaagggtccgaggtacttgtagccaggaagcaccagaccccggccgtcgtcctgcttttgctggttggctttgggcttcggggctccaggtttcagcgcccaccactcgcgaatgccctcagagaggttgtcctcgagccaatctggaagataaccatcggcagccat

SEQ ID NO: 16 - DNA, 9504 bp, Artificial Sequence
  Full length sequence of pV scRS/IRBP hRS vector
agttaattaacacagctgcgcgctcgctcgctcactgaggccgcccgggcaaagcccgggcgtcgggcgacctttggtcgcccggcctcagtgagcgagcgagcgcgcagagagggagtgggggggatccactagttctagagcggccgcaccaccaaatttagcattttcctgagtgaataggtgtgcacatgatgcctagttgctttcaaagaggggaatccatgacattttcatacaattcgagaatgttagtgcttatgtggcaggaaattgttcaaggtcaccccctaaaaaatgatggcgaagaaaggacgaaaacctgagacttctggttgtagttctctccctccattgcttcccttacattaagatagaatgaacagtatggtcgacggcccaggcttcccagcagggctaaggatatgcaaggagtgcattcatccggaggtgttggcagcatcccagccccaccccattctcatcgtaaatcaggctcacttccattggctgcatacggtggagtgatgtgaccatatgtcacttgagcattacacaaatcctaatgagctaaaaatatgtttgttttagctaattgacctctttggccttcataaagcagttggtaaacatcctcagataatgatttccaaagaggtcgaccgaaaagtatcttcctcgcgaactgaatctcagttgatgctagtatcttccatgagacttccttgttgaggcaggtaactctgtgggttaacttgatggggctcagccaaagacctaagaactaaatggattaagatgcttaatgaggccagggctcaacttaatcccctgctcctgggccagctctccagttcagtaaggtagagctttggccgaggacgaggggaagatgtcacgcaagatagaaggctttttgttattacttctctttggctatgaaggtatgtgctattcaaccattgacattcattgcatacttaatacataatttaattaatatcgttgataaataggaatatagcctgaataatataaatattattaattagcaacacgttaattaactaacatgtgttattaatgaacaacagttgtctttgtgtggatggctttccagttctgtgaggagccttctaaagttcaaaggatgcttaaaatccaacagaaaacaggatgggtctcagaaatctataaaatagccagcgatcgcgatttctctttcattaattagattttttctgtctcatccttttgctttagccacattgggattatcgtctaccgaggatgaaggcgaggacccctggtaccaaaaagcatgcaagtgcgattgccaaggaggacccaatgctctgtggtctgcaggtgccacctccttggactgtataccagaatgcccatatcacaagcctctgggtttcgagtcaggggaggtcacaccggaccagatcacctgctctaacccggagcagtatgtgggctggtattcttcgtggactgcaaacaaggcccggctcaacagtcaaggctttgggtgtgcctggctctccaagttccaggacagtagccagtggttacagatagatctgaaggagatcaaagtgatttcagggatcctcacccaggggcgctgtgacatcgatgagtggatgaccaagtacagcgtgcagtacaggaccgatgagcgcctgaactggatttactacaaggaccagactggaaacaaccgggtcttctatggcaactcggaccgcacctccacggttcagaacctgctgcggccccccatcatctcccgcttcatccgcctcatcccgctgggctggcacgtccgcattgccatccggatggagctgctggagtgcgtcagcaagtgtgcctgactcgagagatctaatctcgctttcttgctgtccaatttctattaaaggttcctttgttccctaagtccaactactaaactgggggatattatgaagggccttgagcatctggattctgcctaataaaaaacatttattttcattgcaatgatgtatttaaattatttctgaatattttactaaaaagggaatgtgggaggtcagtgcatttaaaacataaagaaagtagggcgcgccaggaacccctagtgatggagttggccactccctctctgcgcgctcgctcgctcactgaggccgcccgggcaaagcccgggcgtcgggcgacctttggtcgcccggcctcagtgagcgagcgagcgcgcagagagggagtggccaaggccggccaagcttggcgtaatcatggtcatagctgtttcctgtgtgaaattgttatccgctcacaattccacacaacatacgagccggaagcataaagtgtaaagcctggggtgcctaatgagtgagctaactcacattaattgcgttgcgctcactgcccgctttccagtcgggaaacctgtcgtgccagctgcattaatgaatcggccaacgcgcggggagaggcggtttgcgtattgggcgctcttccgctgtcctgcaggacatgtgagcaaaaggccagcaaaaggccaggaaccgtaaaaaggccgcgttgctggcgtttttccataggctccgcccccctgacgagcatcacaaaaatcgacgctcaagtcagaggtggcgaaacccgacaggactataaagataccaggcgtttccccctggaagctccctcgtgcgctctcctgttccgaccctgccgcttaccggatacctgtccgcctttctcccttcgggaagcgtggcgctttctcatagctcacgctgtaggtatctcagttcggtgtaggtcgttcgctccaagctgggctgtgtgcacgaaccccccgttcagcccgaccgctgcgccttatccggtaactatcgtcttgagtccaacccggtaagacacgacttatcgccactggcagcagccactggtaacaggattagcagagcgaggtatgtaggcggtgctacagagttcttgaagtggtggcctaactacggctacactagaaggacagtatttggtatctgcgctctgctgaagccagttaccttcggaaaaagagttggtagctcttgatccggcaaacaaaccaccgctggtagcggtggtttttttgtttgcaagcagcagattacgcgcagaaaaaaaggatctcaagaagatcctttgatcttttctacggggtctgacgctcagtggaacgaaaactcacgttaagggattttggtcatgagattatcaaaaaggatcttcacctagatccttttaaattaaaaatgaagttttaaatcaatctaaagtatatatgagtaaacttggtctgacagttaccaatgcttaatcagtgaggcacctatctcagcgatctgtctatttcgttcatccatagttgcctgactccccgtcgtgtagataactacgatacgggagggcttaccatctggccccagtgctgcaatgataccgcgagacccacgctcaccggctccagatttatcagcaataaaccagccagccggaagggccgagcgcagaagtggtcctgcaactttatccgcctccatccagtctattaattgttgccgggaagctagagtaagtagttcgccagttaatagtttgcgcaacgttgttgccattgctacaggcatcgtggtgtcacgctcgtcgtttggtatggcttcattcagctccggttcccaacgatcaaggcgagttacatgatcccccatgttgtgcaaaaaagcggttagctccttcggtcctccgatcgttgtcagaagtaagttggccgcagtgttatcactcatggttatggcagcactgcataattctcttactgtcatgccatccgtaagatgcttttctgtgactggtgagtactcaaccaagtcattctgagaatagtgtatgcggcgaccgagttgctcttgcccggcgtcaatacgggataataccgcgccacatagcagaactttaaaagtgctcatcattggaaaacgttcttcggggcgaaaactctcaaggatcttaccgctgttgagatccagttcgatgtaacccactcgtgcacccaactgatcttcagcatcttttactttcaccagcgtttctgggtgagcaaaaacaggaaggcaaaatgccgcaaaaaagggaataagggcgacacggaaatgttgaatactcatactcttcctttttcaatattattgaagcatttatcagggttattgtctcatgagcggatacatatttgaatgtatttagaaaaataaacaaataggggttccgcgcacatttccccgaaaagtgccacctgacgtctaagaaaccattattatcatgacattaacctataaaaataggcgtatcacgaggccctttcgtctcgcgcgtttcggtgatgacggtgaaaacctctgacacatgcagctcccggagacggtcacagcttgtctgtaagcggatgccgggagcagacaagcccgtcagggcgcgtcagcgggtgttggcgggtgtcggggctggcttaactatgcggcatcagagcagattgtactgagagtgcaccataaaattgtaaacgttaatattttgttaaaattcgcgttaaatttttgttaaatcagctcattttttaaccaataggccgaaatcggcaaaatcccttataaatcaaaagaatagcccgagatagggttgagtgttgttccagtttggaacaagagtccactattaaagaacgtggactccaacgtcaaagggcgaaaaaccgtctatcagggcgatggcccactacgtgaaccatcacccaaatcaagttttttggggtcgaggtgccgtaaagcactaaatcggaaccctaaagggagcccccgatttagagcttgacggggaaagccggcgaacgtggcgagaaaggaagggaagaaagcgaaaggagcgggcgctagggcgctggcaagtgtagcggtcacgctgcgcgtaaccaccacacccgccgcgcttaatgcgccgctacagggcgcgtactatggttgctttgacgtatgcggtgtgaaataccgcacagatgcgtaaggagaaaataccgcatcaggccgtaacctgtcggatcaccggaaaggacccgtaaagtgataatgattatcatctacatatcacaacgtgcgtggaggccatcaaaccacgtcaaataatcaattatgacgcaggtatcgtattaattgatctgcatcaacttaacgtaaaaacaacttcagacaatacaaatcagcgacactgaatacggggcaacctcatgtcaacgaagaacagaacccgcagaacaacaacccgcaacatccgctttcctaaccaaatgattgaacaaattaacatcgctcttgagcaaaaagggtccgggaatttctcagcctgggtcattgaagcctgccgtcggagactaacgtcagaaaagagagcatatacatcaattaaaagtgatgaagaatgaacatcccgcgttcttccctccgaacaggacgatattgtaaattcacttaattacgagggcattgcagtaattgagttgcagttttaccactttcctgacagtgacagactgcgtgttggctctgtcacagactaaatagtttgaatgattagcagttatggtgatcagtcaaccaccagggaataatccttcatattattatcgtgcttcaccaacgctgcctcaattgctctgaatgcttccagagacaccttatgttctatacatgcaattacaacatcagggtaactcatagaaatggtgctattaagcatattttttacacgaatcagatccacggagggatcatcagcagattgttctttattcattttgtcgctccatgcgcttgctcttcatctagcggttaaaatattacttcaaatctttctgtatgaagatttgagcacgttggccttacatacatctgtcggttgtatttccctccagaatgccagcaggaccgcactttgttacgcaaccaatactattaagtgaaaacattcctaatatttgacataaatcatcaacaaaacacaaggaggtcagaccagattgaaacgataaaaacgataatgcaaactacgcgccctcgtatcacatggaaggttttaccaatggctcaggttgccatttttaaagaaatattcgatcaagtgcgaaaagatttagactgtgaattgttttattctgaactaaaacgtcacaacgtctcacattatatttactatctagccacagataatattcacatcgtgttagaaaacgataacaccgtgttaataaaaggacttaaaaaggttgtaaatgttaaattctcaagaaacacgcatcttatagaaacgtcctatgataggttgaaatcaagagaaatcacatttcagcaatacagggaaaatcttgctaaagcaggagttttccgatgggttacaaatatccatgaacataaaagatattactatacctttgataattcattactatttactgagagcattcagaacactacacaaatctttccacgctaaatcataacgtccggtttcttccgtgtcagcaccggggcgttggcataatgcaatacgtgtacgcgctaaaccctgtgtgcatcgttttaattattcccggacactcccgcagagaagttccccgtcagggctgtggacatagttaatccgggaatacaatgacgattcatcgcacctgacatacattaataaatattaacaatatgaaatttcaactcattgtttagggtttgtttaattttctacacatacgattctgcgaacttcaaaaagcatcgggaataacaccatgaaaaaaatgctactcgctactgcgctggccctgcttattacaggatgtgctcaacagacgtttactgttcaaaacaaaccggcagcagtagcaccaaaggaaaccatcacccatcatttcttcgtttctggaattgggcagaagaaaactgtcgatgcagccaaaatttgtggcggcgcagaaaatgttgttaaaacagaaacccagcaaacattcgtaaatggattgctcggttttattactttaggcatttatactccgctggaagcgcgtgtgtattgctcacaataattgcatgagttgcccatcgatatgggcaactctatctgcactgctcattaatatacttctgggttccttccagttgtttttgcatagtgatcagcctctctctgagggtgaaataatcccgttcagcggtgtctgccagtcggggggaggctgcattatccacgccggaggcggtggtggcttcacgcactgactgacagactgctttgatgtgcaaccgacgacgaccagcggcaacatcatcacgcagagcatcattttcagctttagcatcagctaactccttcgtgtattttgcatcgagcgcagcaacatcacgctgacgcatctgcatgtcagtaattgccgcgttcgccagcttcagttctctggcatttttgtcgcgctgggctttgtaggtaatggcgttatcacggtaatgattaacagcccatgacaggcagacgatgatgcagataaccagagcggagataatcgcggtgactctgctcatacatcaatctctctgaccgttccgcccgcttctttgaattttgcaatcaggctgtcagccttatgctcgaactgaccataaccagcgcccggcagtgaagcccagatattgctgcaacggtcgattgcctgacggatatcaccacgatcaatcataggtaaagcgccacgctccttaatctgctgcaatgccacagcgtcctgacttttcggagagaagtctttcaggccaagctgcttgcggtaggcatcccaccaacgggaaagaagctggtagcgtccggcgcctgttgatttgagttttgggtttagcgtgacaagtttgcgagggtgatcggagtaatcagtaaatagctctccgcctacaatgacgtcataaccatgatttctggttttctgacgtccgttatcagttccctccgaccacgccagcatatcgaggaacgccttacgttgattattgatttctaccatcttctactccggcttttttagcagcgaagcgtttgataagcgaaccaatcgagtcagtaccgatgtagccgataaacacgctcgttatataagcgagattgctacttagtccggcgaagtcgagaaggtcacgaatgaaccaggcgataatggcgcacatcgttgcgtcgattactgtttttgtaaacgcaccgccattatatctgccgcgaaggtacgccattgcaaacgcaaggattgccccgatgccttgttcctttgccgcgagaatggcggccaacaggtcatgtttttctggcatcttcatgtcttacccccaataaggggatttgctctatttaattaggaataaggtcgattactgatagaacaaatccaggctactgtgtttagtaatcagatttgttcgtgaccgatatgcacgggcaaaacggcaggaggttgttagcgcgacctcctgccacccgctttcacgaaggtcatgtgtaaaaggccgcagcgtaactattactaatgaattcaggacagacagtggctacggctcagtttgggttgtgctgttgctgggcggcgatgacgcctgtacgcatttggtgatccggttctgcttccggtattcgcttaattcagcacaacggaaagagcactggctaaccaggctcgccgactcttcacgattatcgactcaatgctcttacctgttgtgcagatataaaaaatcccgaaaccgttatgcaggctctaactattacctgcgaactgtttcgggattgcattttgcagacctctctgcctgcgatggttggagttccagacgatacgtcgaagtgaccaactaggcggaatcggtagtaagcgccgcctcttttcatctcactaccacaacgagcgaattaacccatcgttgagtcaaatttacccaattttattcaataagtcaatatcatgccgttaatatgttgccatccgtggcaatcatgctgctaacgtgtgaccgcattcaaaatgttgtctgcgattgactcttctttgtggcattgcaccaccagagcgtcatacagcggcttaacagtgcgtgaccaggtgggttgggtaaggtttgggattagcatcgtcacagcgcgatatgctgcgcttgctggcatccttgaatagccgacgcctttgcatcttccgcactctttctcgacaactctcccccacagctctgttttggcaatatcaaccgcacggcctgtaccatggcaatctctgcatcttgcccccggcgtcgcggcactacggcaataatccgcataagcgaatgttgcgagcacttgcagtacctttgccttagtatttccttcaagctgcccctgcaggactcg